European Patent Application EP 4 393 499 A1, published July 3, 2024. Title: SMALL EXTRACELLULAR VESICLES WITH ANTIFIBROTIC PROPERTIES. Applicant: FUNDACION PARA LA INVESTIGACION DEL HOSPITAL UNIVERSITARIO Y POLITECNICO LA FE DE LA COMUNIDAD VALENCIANA. The sequence listing filed with the application follows.

SEQUENCE LISTING (4 sequences)

SEQ ID NO: 1 - DNA, 756 bp, Homo sapiens
  source 1..756: mol_type = other DNA
atgggcgtgctgctgacccagaggacactgctgtccctggtgctggccctgctgttcccctctatggcaagcatggcagcaatcggctcctgctctaaggagtaccgcgtgctgctgggccagctgcagaagcagaccgatctgatgcaggacacatccaggctgctggacccctatatccgcatccagggcctggacgtgccaaagctgagggagcactgcagggagaggccaggagcattcccttctgaggagaccctgagaggactgggccggagaggctttctgcagaccctgaacgccacactgggatgcgtgctgcacaggctggcagatctggagcagagactgccaaaggcacaggacctggagcggagcggcctgaacatcgaggatctggagaagctgcagatggccaggcccaatatcctgggcctgcgcaacaatatctactgcatggcccagctgctggataactccgacaccgcagagcctacaaaggcaggaagaggagcatctcagccacctaccccaacaccagcaagcgacgcattccagaggaagctggagggctgtagattcctgcacggctatcaccggtttatgcacagcgtgggcagagtgttttccaagtggggcgagtccccaaataggtctaggggccacagcccacaccaggccctgaggaagggcgtgcggagaacccggccctctagaaagggcaagaggctgatgacaaggggacagctgcctagg

SEQ ID NO: 2 - DNA, 663 bp, Homo sapiens
  source 1..663: mol_type = other DNA
atgggcgtgctgctgacccagaggacactgctgtccctggtgctggccctgctgttcccctctatggcaagcatggcagcaatcggctcctgctctaaggagtaccgcgtgctgctgggccagctgcagaagcagaccgatctgatgcaggacacatccaggctgctggacccctatatccgcatccagggcctggacgtgccaaagctgagggagcactgcagggagaggccaggagcattcccttctgaggagaccctgagaggactgggccggagaggctttctgcagaccctgaacgccacactgggatgcgtgctgcacaggctggcagatctggagcagagactgccaaaggcacaggacctggagcggagcggcctgaacatcgaggatctggagaagctgcagatggccaggcccaatatcctgggcctgcgcaacaatatctactgcatggcccagctgctggataactccgacaccgcagagcctacaaaggcaggaagaggagcatctcagccacctaccccaacaccagcaagcgacgcattccagaggaagctggagggctgtagattcctgcacggctatcaccggtttatgcacagcgtgggcagagtgttttccaagtggggcgagtccccaaataggtctaggggc

SEQ ID NO: 3 - DNA, 1475 bp, Homo sapiens
  source 1..1475: mol_type = other DNA
atgggcgtgctgctgacccagaggacactgctgtccctggtgctggccctgctgttcccctctatggcaagcatggcagcaatcggctcctgctctaaggagtaccgcgtgctgctgggccagctgcagaagcagaccgatctgatgcaggacacatccaggctgctggacccctatatccgcatccagggcctggacgtgccaaagctgagggagcactgcagggagaggccaggagcattcccttctgaggagaccctgagaggactgggccggagaggctttctgcagaccctgaacgccacactgggatgcgtgctgcacaggctggcagatctggagcagagactgccaaaggcacaggacctggagcggagcggcctgaacatcgaggatctggagaagctgcagatggccaggcccaatatcctgggcctgcgcaacaatatctactgcatggcccagctgctggataactccgacaccgcagagcctacaaaggcaggaagaggagcatctcagccacctaccccaacaccagcaagcgacgcattccagaggaagctggagggctgtagattcctgcacggctatcaccggtttatgcacagcgtgggcagagtgttttccaagtggggcgagtccccaaataggtctaggggccacagcccacaccaggccctgaggaagggcgtgcggagaacccggccctctagaaagggcaagaggctgatgacaaggggacagctgcctaggggagtggagggatgcacaaagtgtatcaagtacctgctgttcgtgtttaacttcgtgttttggctggcaggaggcgtgatcctgggagtggccctgtggctgagacacgatccccagaccacaaacctgctgtatctggagctgggcgacaagcccgcccctaataccttttacgtgggcatctatatcctgatcgccgtgggcgccgtgatgatgttcgtgggctttctgggctgctacggcgccatccaggagagccagtgtctgctgggcaccttctttacatgcctggtcatcctgttcgcatgtgaggtggcagcaggaatctggggctttgtgaataaggatcagatcgccaaggacgtgaagcagttctatgatcaggccctgcagcaggccgtggtggacgatgacgccaacaatgccaaggccgtggtgaagacctttcacgagacactggactgctgtggcagctccaccctgacagccctgaccacatccgtgctgaagaacaatctgtgcccctccggctctaacatcatctctaatctgttcaaggaggattgtcaccagaagatcgatgacctgttttctggcaagctgtacctgatcggcatcgccgccatcgtggtggccgtgatcatgatcttcgagatgatcctgtccatggtgctgtgctgtggcatccggaactctagcgtgtattgataagcggccgc

SEQ ID NO: 4 - DNA, 1382 bp, Homo sapiens
  source 1..1382: mol_type = other DNA
atgggcgtgctgctgacccagaggacactgctgtccctggtgctggccctgctgttcccctctatggcaagcatggcagcaatcggctcctgctctaaggagtaccgcgtgctgctgggccagctgcagaagcagaccgatctgatgcaggacacatccaggctgctggacccctatatccgcatccagggcctggacgtgccaaagctgagggagcactgcagggagaggccaggagcattcccttctgaggagaccctgagaggactgggccggagaggctttctgcagaccctgaacgccacactgggatgcgtgctgcacaggctggcagatctggagcagagactgccaaaggcacaggacctggagcggagcggcctgaacatcgaggatctggagaagctgcagatggccaggcccaatatcctgggcctgcgcaacaatatctactgcatggcccagctgctggataactccgacaccgcagagcctacaaaggcaggaagaggagcatctcagccacctaccccaacaccagcaagcgacgcattccagaggaagctggagggctgtagattcctgcacggctatcaccggtttatgcacagcgtgggcagagtgttttccaagtggggcgagtccccaaataggtctaggggcggagtggagggatgcacaaagtgtatcaagtacctgctgttcgtgtttaacttcgtgttttggctggcaggaggcgtgatcctgggagtggccctgtggctgagacacgatccccagaccacaaacctgctgtatctggagctgggcgacaagcccgcccctaataccttttacgtgggcatctatatcctgatcgccgtgggcgccgtgatgatgttcgtgggctttctgggctgctacggcgccatccaggagagccagtgtctgctgggcaccttctttacatgcctggtcatcctgttcgcatgtgaggtggcagcaggaatctggggctttgtgaataaggatcagatcgccaaggacgtgaagcagttctatgatcaggccctgcagcaggccgtggtggacgatgacgccaacaatgccaaggccgtggtgaagacctttcacgagacactggactgctgtggcagctccaccctgacagccctgaccacatccgtgctgaagaacaatctgtgcccctccggctctaacatcatctctaatctgttcaaggaggattgtcaccagaagatcgatgacctgttttctggcaagctgtacctgatcggcatcgccgccatcgtggtggccgtgatcatgatcttcgagatgatcctgtccatggtgctgtgctgtggcatccggaactctagcgtgtattgataagcggccgc